European Patent Specification EP 3 452 591 B1, published August 16, 2023. Title: MACROMOLECULE ANAYSIS EMPLOYING NUCLEIC ACID ENCODING. Applicant: ProCure Life Sciences Inc. Chee, Mark Gunderson, Kevin Weiner, Michael Phillip. Application PCT. The sequence listing filed with the application follows.

SEQUENCE LISTING (180 sequences)

SEQ ID NO: 1 - DNA, 15 bp, Artificial Sequence
  oligonucleotide barcode BC_1
atgtctagcatgccg

SEQ ID NO: 2 - DNA, 15 bp, Artificial Sequence
  oligonucleotide barcode BC_2
ccgtgtcatgtggaa

SEQ ID NO: 3 - DNA, 15 bp, Artificial Sequence
  oligonucleotide barcode BC_3
taagccggtatatca

SEQ ID NO: 4 - DNA, 15 bp, Artificial Sequence
  oligonucleotide barcode BC_4
ttcgatatgacggaa

SEQ ID NO: 5 - DNA, 15 bp, Artificial Sequence
  oligonucleotide barcode BC_5
cgtatacgcgttagg

SEQ ID NO: 6 - DNA, 15 bp, Artificial Sequence
  oligonucleotide barcode BC_6
aactgccgagattcc

SEQ ID NO: 7 - DNA, 15 bp, Artificial Sequence
  oligonucleotide barcode BC_7
tgatcttagctgtgc

SEQ ID NO: 8 - DNA, 15 bp, Artificial Sequence
  oligonucleotide barcode BC_8
gagtcggtaccttga

SEQ ID NO: 9 - DNA, 15 bp, Artificial Sequence
  oligonucleotide barcode BC_9
ccgcttgtgatctgg

SEQ ID NO: 10 - DNA, 15 bp, Artificial Sequence
  oligonucleotide barcode BC_10
agatagcgtaccgga

SEQ ID NO: 11 - DNA, 15 bp, Artificial Sequence
  oligonucleotide barcode BC_11
tccaggctcatcatc

SEQ ID NO: 12 - DNA, 15 bp, Artificial Sequence
  oligonucleotide barcode BC_12
gagtactagagccaa

SEQ ID NO: 13 - DNA, 15 bp, Artificial Sequence
  oligonucleotide barcode BC_13
gagcgtcaataacgg

SEQ ID NO: 14 - DNA, 15 bp, Artificial Sequence
  oligonucleotide barcode BC_14
gcggtatctacactg

SEQ ID NO: 15 - DNA, 15 bp, Artificial Sequence
  oligonucleotide barcode BC_15
cttctccgaagagaa

SEQ ID NO: 16 - DNA, 15 bp, Artificial Sequence
  oligonucleotide barcode BC_16
tgaagcctgtgttaa

SEQ ID NO: 17 - DNA, 15 bp, Artificial Sequence
  oligonucleotide barcode BC_17
ctggatggttgtcga

SEQ ID NO: 18 - DNA, 15 bp, Artificial Sequence
  oligonucleotide barcode BC_18
actgcacggttccaa

SEQ ID NO: 19 - DNA, 15 bp, Artificial Sequence
  oligonucleotide barcode BC_19
cgagagatggtcctt

SEQ ID NO: 20 - DNA, 15 bp, Artificial Sequence
  oligonucleotide barcode BC_20
tcttgagagacaaga

SEQ ID NO: 21 - DNA, 15 bp, Artificial Sequence
  oligonucleotide barcode BC_21
aattcgcactgtgtt

SEQ ID NO: 22 - DNA, 15 bp, Artificial Sequence
  oligonucleotide barcode BC_22
gtagtgccgctaaga

SEQ ID NO: 23 - DNA, 15 bp, Artificial Sequence
  oligonucleotide barcode BC_23
cctatagcacaatcc

SEQ ID NO: 24 - DNA, 15 bp, Artificial Sequence
  oligonucleotide barcode BC_24
atcaccgaggttgga

SEQ ID NO: 25 - DNA, 15 bp, Artificial Sequence
  oligonucleotide barcode BC_25
gattcaacggagaag

SEQ ID NO: 26 - DNA, 15 bp, Artificial Sequence
  oligonucleotide barcode BC_26
acgaacctcgcacca

SEQ ID NO: 27 - DNA, 15 bp, Artificial Sequence
  oligonucleotide barcode BC_27
aggacttcaagaaga

SEQ ID NO: 28 - DNA, 15 bp, Artificial Sequence
  oligonucleotide barcode BC_28
ggttgaatcctcgca

SEQ ID NO: 29 - DNA, 15 bp, Artificial Sequence
  oligonucleotide barcode BC_29
aaccaacctctagcg

SEQ ID NO: 30 - DNA, 15 bp, Artificial Sequence
  oligonucleotide barcode BC_30
acgcgaatatctaac

SEQ ID NO: 31 - DNA, 15 bp, Artificial Sequence
  oligonucleotide barcode BC_31
gttgagaattacacc

SEQ ID NO: 32 - DNA, 15 bp, Artificial Sequence
  oligonucleotide barcode BC_32
ctctctctgtgaacc

SEQ ID NO: 33 - DNA, 15 bp, Artificial Sequence
  oligonucleotide barcode BC_33
gccatcagtaagaga

SEQ ID NO: 34 - DNA, 15 bp, Artificial Sequence
  oligonucleotide barcode BC_34
gcaacgtgaattgag

SEQ ID NO: 35 - DNA, 15 bp, Artificial Sequence
  oligonucleotide barcode BC_35
ctaagtagagccaca

SEQ ID NO: 36 - DNA, 15 bp, Artificial Sequence
  oligonucleotide barcode BC_36
tgtctgttggaagcg

SEQ ID NO: 37 - DNA, 15 bp, Artificial Sequence
  oligonucleotide barcode BC_37
ttaatagacagcgcg

SEQ ID NO: 38 - DNA, 15 bp, Artificial Sequence
  oligonucleotide barcode BC_38
cgacgctctaacaag

SEQ ID NO: 39 - DNA, 15 bp, Artificial Sequence
  oligonucleotide barcode BC_39
catggcttattgaga

SEQ ID NO: 40 - DNA, 15 bp, Artificial Sequence
  oligonucleotide barcode BC_40
actaggtatggccgg

SEQ ID NO: 41 - DNA, 15 bp, Artificial Sequence
  oligonucleotide barcode BC_41
gtcctcgtctatcct

SEQ ID NO: 42 - DNA, 15 bp, Artificial Sequence
  oligonucleotide barcode BC_42
taggattccgttacc

SEQ ID NO: 43 - DNA, 15 bp, Artificial Sequence
  oligonucleotide barcode BC_43
tctgaccaccggaag

SEQ ID NO: 44 - DNA, 15 bp, Artificial Sequence
  oligonucleotide barcode BC_44
agagtcacctcgtgg

SEQ ID NO: 45 - DNA, 15 bp, Artificial Sequence
  oligonucleotide barcode BC_45
ctgatgtagtcgaag

SEQ ID NO: 46 - DNA, 15 bp, Artificial Sequence
  oligonucleotide barcode BC_46
gtcggttgcggatag

SEQ ID NO: 47 - DNA, 15 bp, Artificial Sequence
  oligonucleotide barcode BC_47
tcctcctcctaagaa

SEQ ID NO: 48 - DNA, 15 bp, Artificial Sequence
  oligonucleotide barcode BC_48
attcggtccacttca

SEQ ID NO: 49 - DNA, 15 bp, Artificial Sequence
  oligonucleotide barcode BC_49
ccttacaggtctgcg

SEQ ID NO: 50 - DNA, 15 bp, Artificial Sequence
  oligonucleotide barcode BC_50
gatcattggccaatt

SEQ ID NO: 51 - DNA, 15 bp, Artificial Sequence
  oligonucleotide barcode BC_51
ttcaaggctgagttg

SEQ ID NO: 52 - DNA, 15 bp, Artificial Sequence
  oligonucleotide barcode BC_52
tggctcgattgaatc

SEQ ID NO: 53 - DNA, 15 bp, Artificial Sequence
  oligonucleotide barcode BC_53
gtaagccatccgctc

SEQ ID NO: 54 - DNA, 15 bp, Artificial Sequence
  oligonucleotide barcode BC_54
acacatgcgtagaca

SEQ ID NO: 55 - DNA, 15 bp, Artificial Sequence
  oligonucleotide barcode BC_55
tgctatggattcaag

SEQ ID NO: 56 - DNA, 15 bp, Artificial Sequence
  oligonucleotide barcode BC_56
ccacgaggcttagtt

SEQ ID NO: 57 - DNA, 15 bp, Artificial Sequence
  oligonucleotide barcode BC_57
ggccaactaaggtgc

SEQ ID NO: 58 - DNA, 15 bp, Artificial Sequence
  oligonucleotide barcode BC_58
gcacctattcgacaa

SEQ ID NO: 59 - DNA, 15 bp, Artificial Sequence
  oligonucleotide barcode BC_59
tggacacgatcggct

SEQ ID NO: 60 - DNA, 15 bp, Artificial Sequence
  oligonucleotide barcode BC_60
ctataattccaacgg

SEQ ID NO: 61 - DNA, 15 bp, Artificial Sequence
  oligonucleotide barcode BC_61
aacgtggttagtaag

SEQ ID NO: 62 - DNA, 15 bp, Artificial Sequence
  oligonucleotide barcode BC_62
caaggaacgagtggc

SEQ ID NO: 63 - DNA, 15 bp, Artificial Sequence
  oligonucleotide barcode BC_63
caccagaacggaaga

SEQ ID NO: 64 - DNA, 15 bp, Artificial Sequence
  oligonucleotide barcode BC_64
cgtacggtcaagcaa

SEQ ID NO: 65 - DNA, 15 bp, Artificial Sequence
  oligonucleotide barcode BC_65
tcggtgacaggctaa

SEQ ID NO: 66 - DNA, 15 bp, Artificial Sequence
  oligonucleotide barcode BC_1 REV
cggcatgctagacat

SEQ ID NO: 67 - DNA, 15 bp, Artificial Sequence
  oligonucleotide barcode BC_2  REV
ttccacatgacacgg

SEQ ID NO: 68 - DNA, 15 bp, Artificial Sequence
  oligonucleotide barcode BC_3  REV
tgatataccggctta

SEQ ID NO: 69 - DNA, 15 bp, Artificial Sequence
  oligonucleotide barcode BC_4  REV
ttccgtcatatcgaa

SEQ ID NO: 70 - DNA, 15 bp, Artificial Sequence
  oligonucleotide barcode BC_5  REV
cctaacgcgtatacg

SEQ ID NO: 71 - DNA, 15 bp, Artificial Sequence
  oligonucleotide barcode BC_6  REV
ggaatctcggcagtt

SEQ ID NO: 72 - DNA, 15 bp, Artificial Sequence
  oligonucleotide barcode BC_7  REV
gcacagctaagatca

SEQ ID NO: 73 - DNA, 15 bp, Artificial Sequence
  oligonucleotide barcode BC_8  REV
tcaaggtaccgactc

SEQ ID NO: 74 - DNA, 15 bp, Artificial Sequence
  oligonucleotide barcode BC_9  REV
ccagatcacaagcgg

SEQ ID NO: 75 - DNA, 15 bp, Artificial Sequence
  oligonucleotide barcode BC_10  REV
tccggtacgctatct

SEQ ID NO: 76 - DNA, 15 bp, Artificial Sequence
  oligonucleotide barcode BC_11  REV
gatgatgagcctgga

SEQ ID NO: 77 - DNA, 15 bp, Artificial Sequence
  oligonucleotide barcode BC_12  REV
ttggctctagtactc

SEQ ID NO: 78 - DNA, 15 bp, Artificial Sequence
  oligonucleotide barcode BC_13  REV
ccgttattgacgctc

SEQ ID NO: 79 - DNA, 15 bp, Artificial Sequence
  oligonucleotide barcode BC_14  REV
cagtgtagataccgc

SEQ ID NO: 80 - DNA, 15 bp, Artificial Sequence
  oligonucleotide barcode BC_15  REV
ttctcttcggagaag

SEQ ID NO: 81 - DNA, 15 bp, Artificial Sequence
  oligonucleotide barcode BC_16  REV
ttaacacaggcttca

SEQ ID NO: 82 - DNA, 15 bp, Artificial Sequence
  oligonucleotide barcode BC_17  REV
tcgacaaccatccag

SEQ ID NO: 83 - DNA, 15 bp, Artificial Sequence
  oligonucleotide barcode BC_18  REV
ttggaaccgtgcagt

SEQ ID NO: 84 - DNA, 15 bp, Artificial Sequence
  oligonucleotide barcode BC_19 REV
aaggaccatctctcg

SEQ ID NO: 85 - DNA, 15 bp, Artificial Sequence
  oligonucleotide barcode BC_20 REV
tcttgtctctcaaga

SEQ ID NO: 86 - DNA, 15 bp, Artificial Sequence
  oligonucleotide barcode BC_21 REV
aacacagtgcgaatt

SEQ ID NO: 87 - DNA, 15 bp, Artificial Sequence
  oligonucleotide barcode BC_22 REV
tcttagcggcactac

SEQ ID NO: 88 - DNA, 15 bp, Artificial Sequence
  oligonucleotide barcode BC_23 REV
ggattgtgctatagg

SEQ ID NO: 89 - DNA, 15 bp, Artificial Sequence
  oligonucleotide barcode BC_24 REV
tccaacctcggtgat

SEQ ID NO: 90 - DNA, 15 bp, Artificial Sequence
  oligonucleotide barcode BC_25 REV
cttctccgttgaatc

SEQ ID NO: 91 - DNA, 15 bp, Artificial Sequence
  oligonucleotide barcode BC_26 REV
tggtgcgaggttcgt

SEQ ID NO: 92 - DNA, 15 bp, Artificial Sequence
  oligonucleotide barcode BC_27 REV
tcttcttgaagtcct

SEQ ID NO: 93 - DNA, 15 bp, Artificial Sequence
  oligonucleotide barcode BC_28 REV
tgcgaggattcaacc

SEQ ID NO: 94 - DNA, 15 bp, Artificial Sequence
  oligonucleotide barcode BC_29 REV
cgctagaggttggtt

SEQ ID NO: 95 - DNA, 15 bp, Artificial Sequence
  oligonucleotide barcode BC_30 REV
gttagatattcgcgt

SEQ ID NO: 96 - DNA, 15 bp, Artificial Sequence
  oligonucleotide barcode BC_31 REV
ggtgtaattctcaac

SEQ ID NO: 97 - DNA, 15 bp, Artificial Sequence
  oligonucleotide barcode BC_32 REV
ggttcacagagagag

SEQ ID NO: 98 - DNA, 15 bp, Artificial Sequence
  oligonucleotide barcode BC_33 REV
tctcttactgatggc

SEQ ID NO: 99 - DNA, 15 bp, Artificial Sequence
  oligonucleotide barcode BC_34 REV
ctcaattcacgttgc

SEQ ID NO: 100 - DNA, 15 bp, Artificial Sequence
  oligonucleotide barcode BC_35 REV
tgtggctctacttag

SEQ ID NO: 101 - DNA, 15 bp, Artificial Sequence
  oligonucleotide barcode BC_36 REV
cgcttccaacagaca

SEQ ID NO: 102 - DNA, 15 bp, Artificial Sequence
  oligonucleotide barcode BC_37 REV
cgcgctgtctattaa

SEQ ID NO: 103 - DNA, 15 bp, Artificial Sequence
  oligonucleotide barcode BC_38 REV
cttgttagagcgtcg

SEQ ID NO: 104 - DNA, 15 bp, Artificial Sequence
  oligonucleotide barcode BC_39 REV
tctcaataagccatg

SEQ ID NO: 105 - DNA, 15 bp, Artificial Sequence
  oligonucleotide barcode BC_40 REV
ccggccatacctagt

SEQ ID NO: 106 - DNA, 15 bp, Artificial Sequence
  oligonucleotide barcode BC_41 REV
aggatagacgaggac

SEQ ID NO: 107 - DNA, 15 bp, Artificial Sequence
  oligonucleotide barcode BC_42 REV
ggtaacggaatccta

SEQ ID NO: 108 - DNA, 15 bp, Artificial Sequence
  oligonucleotide barcode BC_43 REV
cttccggtggtcaga

SEQ ID NO: 109 - DNA, 15 bp, Artificial Sequence
  oligonucleotide barcode BC_44 REV
ccacgaggtgactct

SEQ ID NO: 110 - DNA, 15 bp, Artificial Sequence
  oligonucleotide barcode BC_45 REV
cttcgactacatcag

SEQ ID NO: 111 - DNA, 15 bp, Artificial Sequence
  oligonucleotide barcode BC_46 REV
ctatccgcaaccgac

SEQ ID NO: 112 - DNA, 15 bp, Artificial Sequence
  oligonucleotide barcode BC_47 REV
ttcttaggaggagga

SEQ ID NO: 113 - DNA, 15 bp, Artificial Sequence
  oligonucleotide barcode BC_48 REV
tgaagtggaccgaat

SEQ ID NO: 114 - DNA, 15 bp, Artificial Sequence
  oligonucleotide barcode BC_49 REV
cgcagacctgtaagg

SEQ ID NO: 115 - DNA, 15 bp, Artificial Sequence
  oligonucleotide barcode BC_50 REV
aattggccaatgatc

SEQ ID NO: 116 - DNA, 15 bp, Artificial Sequence
  oligonucleotide barcode BC_51 REV
caactcagccttgaa

SEQ ID NO: 117 - DNA, 15 bp, Artificial Sequence
  oligonucleotide barcode BC_52 REV
gattcaatcgagcca

SEQ ID NO: 118 - DNA, 15 bp, Artificial Sequence
  oligonucleotide barcode BC_53 REV
gagcggatggcttac

SEQ ID NO: 119 - DNA, 15 bp, Artificial Sequence
  oligonucleotide barcode BC_54 REV
tgtctacgcatgtgt

SEQ ID NO: 120 - DNA, 15 bp, Artificial Sequence
  oligonucleotide barcode BC_55 REV
cttgaatccatagca

SEQ ID NO: 121 - DNA, 15 bp, Artificial Sequence
  oligonucleotide barcode BC_56 REV
aactaagcctcgtgg

SEQ ID NO: 122 - DNA, 15 bp, Artificial Sequence
  oligonucleotide barcode BC_57 REV
gcaccttagttggcc

SEQ ID NO: 123 - DNA, 15 bp, Artificial Sequence
  oligonucleotide barcode BC_58 REV
ttgtcgaataggtgc

SEQ ID NO: 124 - DNA, 15 bp, Artificial Sequence
  oligonucleotide barcode BC_59 REV
agccgatcgtgtcca

SEQ ID NO: 125 - DNA, 15 bp, Artificial Sequence
  oligonucleotide barcode BC_60 REV
ccgttggaattatag

SEQ ID NO: 126 - DNA, 15 bp, Artificial Sequence
  oligonucleotide barcode BC_61 REV
cttactaaccacgtt

SEQ ID NO: 127 - DNA, 15 bp, Artificial Sequence
  oligonucleotide barcode BC_62 REV
gccactcgttccttg

SEQ ID NO: 128 - DNA, 15 bp, Artificial Sequence
  oligonucleotide barcode BC_63 REV
tcttccgttctggtg

SEQ ID NO: 129 - DNA, 15 bp, Artificial Sequence
  oligonucleotide barcode BC_64 REV
ttgcttgaccgtacg

SEQ ID NO: 130 - DNA, 15 bp, Artificial Sequence
  oligonucleotide barcode BC_65 REV
ttagcctgtcaccga

SEQ ID NO: 131 - protein, 16 aa, Artificial Sequence
  synthetic peptide
  MOD_RES 1: formyl-Methionine
MDVEAWLGARVPLVET

SEQ ID NO: 132 - protein, 10 aa, Artificial Sequence
  synthetic peptide
TENLYFQNHV

SEQ ID NO: 133 - DNA, 20 bp, Artificial Sequence
  oligonucleotide primer
aatgatacggcgaccaccga

SEQ ID NO: 134 - DNA, 24 bp, Artificial Sequence
  oligonucleotide primer
caagcagaagacggcatacgagat

SEQ ID NO: 135 - DNA, 5 bp, Artificial Sequence
  oligonucleotide
  misc_feature (1)...(5): n = A,T,C or G
nnnnn

SEQ ID NO: 136 - protein, 8 aa, Artificial Sequence
  synthetic peptide
DYKDDDDK

SEQ ID NO: 137 - protein, 14 aa, Artificial Sequence
  synthetic peptide
GKPIPNPLLGLDST

SEQ ID NO: 138 - protein, 10 aa, Artificial Sequence
  synthetic peptide
EQKLISEEDL

SEQ ID NO: 139 - protein, 9 aa, Artificial Sequence
  synthetic peptide
YPYDVPDYA

SEQ ID NO: 140 - protein, 9 aa, Artificial Sequence
  synthetic peptide
NWSHPQFEK

SEQ ID NO: 141 - DNA, 82 bp, Artificial Sequence
  synthetic oligonucleotide
  modified_base 1: biotin
tttttgcaaatggcattctgacatcccgtagtccgcgacactagatgtctagcatgccgccgtgtcatgtggaaactgagtg

SEQ ID NO: 142 - DNA, 72 bp, Artificial Sequence
  synthetic oligonucleotide
  modified_base 1: biotin
ttttttttttgactggttccaattgacaagccgtagtccgcgacactagtaagccggtatatcaactgagtg

SEQ ID NO: 143 - DNA, 10 bp, Artificial Sequence
  synthetic oligonucleotide
  modified_base 1: biotin
  modified_base 10: three carbon (3C) spacer
tttttttttt

SEQ ID NO: 144 - DNA, 62 bp, Artificial Sequence
  synthetic oligonucleotide
  modified_base (31)...(32): 18-atom hexa-ethyleneglycol spacer
  modified_base 62: three carbon (3C) spacer
ggatgtcagaatgccatttgcttttttttttcactcagtcctaacgcgtatacgcactcagt

SEQ ID NO: 145 - DNA, 63 bp, Artificial Sequence
  synthetic oligonucleotide
  modified_base (31)...(32): 18-atom hexa-ethyleneglycol spacer
  modified_base 63: three carbon (3C) spacer
ggatgtcagaatgccatttgcttttttttttcactcagtcctaacgcgtatacgtcactcagt

SEQ ID NO: 146 - DNA, 63 bp, Artificial Sequence; identical to SEQ ID NO: 145
  synthetic oligonucleotide
  modified_base (31)...(32): five 18-atom hexa-ethyleneglycol spacers
  modified_base 63: three carbon (3C) spacer

SEQ ID NO: 147 - DNA, 71 bp, Artificial Sequence
  synthetic oligonucleotide
  modified_base (25)...(26): 18-atom hexa-ethyleneglycol spacer
  modified_base 63: three carbon (3C) spacer)
gcttgtcaattggaaccagtcttttcactcagtcctaacgcgtatacgggaatctcggcagttcactcagt

SEQ ID NO: 148 - DNA, 44 bp, Artificial Sequence
  synthetic oligonucleotide
  modified_base 44: three carbon (3C) spacer
cgatttgcaaggatcactcgtcactcagtcctaacgcgtatacg

SEQ ID NO: 149 - DNA, 8 bp, Artificial Sequence
  spacer sequence
actgagtg

SEQ ID NO: 150 - DNA, 8 bp, Artificial Sequence
  spacer sequence
cactcagt

SEQ ID NO: 151 - DNA, 18 bp, Artificial Sequence
  oligonucleotide primer
cgtagtccgcgacactag

SEQ ID NO: 152 - DNA, 20 bp, Artificial Sequence
  oligonucleotide primer
cgatttgcaaggatcactcg

SEQ ID NO: 153 - DNA, 21 bp, Artificial Sequence
  synthetic oligonucleotide
gcaaatggcattctgacatcc

SEQ ID NO: 154 - DNA, 21 bp, Artificial Sequence
  synthetic oligonucleotide
gactggttccaattgacaagc

SEQ ID NO: 155 - DNA, 23 bp, Artificial Sequence
  synthetic oligonucleotide
  modified_base 23: three carbon (3C) spacer
cgtatacgcgttaggactgagtg

SEQ ID NO: 156 - DNA, 38 bp, Artificial Sequence
  synthetic oligonucleotide
  modified_base 38: three carbon (3C) spacer
aactgccgagattcccgtatacgcgttaggactgagtg

SEQ ID NO: 157 - DNA, 46 bp, Artificial Sequence
  oligonucleotide primer
agtccgcgcaatcagatgtctagcatgccggatccggatcgatctc

SEQ ID NO: 158 - DNA, 46 bp, Artificial Sequence
  oligonucleotide primer
agtccgcgcaatcagccgtgtcatgtggaagatccggatcgatctc

SEQ ID NO: 159 - DNA, 46 bp, Artificial Sequence
  oligonucleotide primer
agtccgcgcaatcagtaagccggtatatcagatccggatcgatctc

SEQ ID NO: 160 - DNA, 46 bp, Artificial Sequence
  oligonucleotide primer
agtccgcgcaatcagttcgatatgacggaagatccggatcgatctc

SEQ ID NO: 161 - DNA, 46 bp, Artificial Sequence
  oligonucleotide primer
tgcaaggatcactcgccagatcacaagcgggagatcgatccggatc

SEQ ID NO: 162 - DNA, 46 bp, Artificial Sequence
  oligonucleotide primer
tgcaaggatcactcgtccggtacgctatctgagatcgatccggatc

SEQ ID NO: 163 - DNA, 46 bp, Artificial Sequence
  oligonucleotide primer
tgcaaggatcactcggatgatgagcctggagagatcgatccggatc

SEQ ID NO: 164 - DNA, 46 bp, Artificial Sequence
  oligonucleotide primer
tgcaaggatcactcgttggctctagtactcgagatcgatccggatc

SEQ ID NO: 165 - DNA, 21 bp, Artificial Sequence
  oligonucleotide primer
aatcgtagtccgcgcaatcag

SEQ ID NO: 166 - DNA, 21 bp, Artificial Sequence
  oligonucleotide primer
acgatttgcaaggatcactcg

SEQ ID NO: 167 - DNA, 16 bp, Artificial Sequence
  spacer sequence
gatccggatcgatctc

SEQ ID NO: 168 - DNA, 734 bp, Artificial Sequence
  extended recording tag construct
aatcacggtacaagtcactcatccgtacgctatctgagaatcgtccagatccggcatgctagtatctggtgcagactacgattgttacagatcactcagatgatgagcacagaaaatcgtcgaatcttccatcaccatcgaacagttacgattaatgtagtccgcacaatcgaatgtctaacatgccgaatcccggacgtctccagcttctaaaccaacagtagtcgcacaaatcattgtacggtacaagatctaacgagagatgatcggatctgaccactttaaacactgattacgcagactacgattacgatttaagaatcctcgtccggtacaatcatagtccgcacaatcaaccgtgtcatgtgaagatcagatcgatctcgaatagcgtaccagacagtgatcttgcaaatcgtaatgtgtccgcgccaatcgatagccatgaatcccagtcgatctcccgcttgtgatctggcgatcgccttgtaccgtcgtacgatttgagatcacctcgttaactcaagctaaagatcgtccggatcgctttataaacatctgattgcgcggtacgattatcgtagtccgcacatatcgaacctgttgaagatccggatcgtctctccaggctcatcatccgagtgatccttgcaaataatcatgtccgcaccatcaggtgtctaacgcttgccggatccgaatcgatctctccaggctcatcatcgaagtgatgt

SEQ ID NO: 169 - protein, 10 aa, Artificial Sequence
  synthetic peptide
CPVQLWVDST

SEQ ID NO: 170 - protein, 10 aa, Artificial Sequence
  synthetic peptide
  VARIANT (1)...(10): Xaa = Any Amino Acid
CPXQXWXDXT

SEQ ID NO: 171 - protein, 8 aa, Artificial Sequence
  FLAG epitope peptide
DYKDDDDK

SEQ ID NO: 172 - protein, 14 aa, Artificial Sequence
  V5 epitope peptide
GKPIPNPLLGLDST

SEQ ID NO: 173 - protein, 10 aa, Artificial Sequence
  c-Myc epitope peptide
EQKLISEEDL

SEQ ID NO: 174 - protein, 9 aa, Artificial Sequence
  HA epitope peptide
YPYDVPDYA

SEQ ID NO: 175 - protein, 14 aa, Artificial Sequence
  V5 epitope peptide
GKPIPNPLLGLDST

SEQ ID NO: 176 - protein, 9 aa, Artificial Sequence
  StrepTag II peptide
NWSHPQFEK

SEQ ID NO: 177 - DNA, 36 bp, Artificial Sequence
  synthetic nucloetide
  misc_feature (11)...(22): compartment bar code n = A, C, T, or G
  misc_feature (23)...(27): unique molecular identifier n = A, T, C or G
gcgcaatcagnnnnnnnnnnnnnnnnntgcaaggat

SEQ ID NO: 178 - DNA, 12 bp, Artificial Sequence
  synthetic nucloetide
  misc_feature (1)...(12): Compartment barcod n = A, T, C or G
nnnnnnnnnnnn

SEQ ID NO: 179 - DNA, 5 bp, Artificial Sequence
  synthetic nucloetide
  misc_feature (1)...(5): Unique molecular identifier; n = A, T, C or G
nnnnn

SEQ ID NO: 180 - protein, 10 aa, Artificial Sequence
  butelase I peptide substrate
CGGSSGSNHV